European Patent Application EP 4 215 201 A1, published July 26, 2023. Title: NOVEL RECOMBINANT ADENO-ASSOCIATED VIRAL VECTORS RESTRICTING OFF-TARGET TRANSDUCTION IN LIVER AND USES THEREOF. Applicant: Ohio State Innovation Foundation. Application EP. The sequence listing filed with the application follows.

SEQUENCE LISTING (1 sequence)

SEQ ID NO: 1 - DNA, 19 bp, synthetic construct
  source 1..19: mol_type = other DNA
ctatgtggacgctgcttta